European Patent Application EP 4 410 828 A1, published August 7, 2024. Title: Oligonucleotide encoding a tissue inhibitor of metalloproteases protein for medical use in mammals. Applicant: Eberhard Karls Universität Tübingen Medizinische Fakultät. Application EP. The sequence listing filed with the application follows.

SEQUENCE LISTING (5 sequences)

SEQ ID NO: 1 - protein, 207 aa, synthetic construct
MAPFEPLASGILLLLWLIAPSRACTCVPPHPQTAFCNSDLVIRAKFVGTPEVNQTTLYQRYEIKMTKMYKGFQALGDAADIRFVYTPAMESVCGYFHRSHNRSEEFLIAGKLQDGLLHITTCSFVAPWNSLSLAQRRGFTKTYTVGCEECTVFPCLSIPCKLQSGTHCLWTDQLLQGSEKGFQSRHLACLPREPGLCTWQSLRSQIA

SEQ ID NO: 2 - RNA, 624 nt, synthetic construct
  source 1..624: mol_type = other RNA
atggctccctttgaaccccttgcttcaggcatactgctgcttctgtggctcattgcccctagcagagcatgcacatgtgtgccaccacatccacagaccgctttctgcaacagcgacctggtaatcagggcgaagtttgtcggtactcctgaagtgaaccagacgaccctctatcagcgctatgagatcaagatgaccaagatgtacaagggctttcaagcactgggtgatgctgcagacatccgcttcgtctatactcctgcgatggagtctgtgtgtggctacttccacaggtcccataatcggtccgaagagttcctgattgccggcaaactgcaggatggactcctccacatcactacatgcagcttcgttgccccatggaattccctgagtctggcccaacgtagagggttcacgaaaacctacaccgttgggtgtgaggagtgtaccgtgtttccctgcttgagcattccgtgcaaactccagtctggaacacactgtctgtggactgaccagctgctgcaaggatcagagaagggctttcagagtcggcatttggcctgcttgcctagagaacccgggctttgcacatggcagtctctgcgaagccagatagcctga

SEQ ID NO: 3 - DNA, 558 bp, synthetic construct
  source 1..558: mol_type = other DNA
atgggagtcaaagttctgtttgccctgatctgcatcgctgtggccgaggccaagcccaccgagaacaacgaagacttcaacatcgtggccgtggccagcaacttcgcgaccacggatctcgatgctgaccgcgggaagttgcccggcaagaagctgccgctggaggtgctcaaagagatggaagccaatgcccggaaagctggctgcaccaggggctgtctgatctgcctgtcccacatcaagtgcacgcccaagatgaagaagttcatcccaggacgctgccacacctacgaaggcgacaaagagtccgcacagggcggcataggcgaggcgatcgtcgacattcctgagattcctgggttcaaggacttggagcctatggagcagttcatcgcacaggtcgatctgtgtgtggactgcacaactggctgcctcaaagggcttgccaacgtgcagtgttctgacctgctcaagaagtggctgccgcaacgctgtgcgacctttgccagcaagatccagggccaggtggacaagatcaagggggccggtggtgactaa

SEQ ID NO: 4 - DNA, 27 bp, synthetic construct
  source 1..27: mol_type = other DNA
ttggaccctcgtacagaagctaatacg

SEQ ID NO: 5 - DNA, 149 bp, synthetic construct
  source 1..149: mol_type = other DNA
ttttttttttttttttttttttttttttttttttttttttttttttttttttttttttttttttttttttttttttttttttttttttttttttttttttttttttttttttttttttttcttcctactcaggctttattcaaagacca